European Patent Application EP 4 603 500 A1, published August 20, 2025. Title: Peptide Having Activity of Promoting Hair Growth and Inhibiting Hair Loss and Uses Thereof. Applicant: CAREGENE CO., LTD. Application KR. The sequence listing filed with the application follows.

SEQUENCE LISTING (13 sequences)

SEQ ID NO: 1 - protein, 10 aa, synthetic construct
ASKVKVSMKF

SEQ ID NO: 2 - DNA, 20 bp, synthetic construct
  source 1..20: mol_type = other DNA
ccagctattgtaacacctca

SEQ ID NO: 3 - DNA, 20 bp, synthetic construct
  source 1..20: mol_type = other DNA
ttcagatgtaggcagctgtc

SEQ ID NO: 4 - DNA, 28 bp, synthetic construct
  source 1..28: mol_type = other DNA
accttcgttgccctctgtgccacagatg

SEQ ID NO: 5 - DNA, 21 bp, synthetic construct
  source 1..21: mol_type = other DNA
aggcccggaggcagtccgggt

SEQ ID NO: 6 - DNA, 20 bp, synthetic construct
  source 1..20: mol_type = other DNA
ggagccaaaagggtcatcat

SEQ ID NO: 7 - DNA, 20 bp, synthetic construct
  source 1..20: mol_type = other DNA
gtgatggcatggactgtggt

SEQ ID NO: 8 - DNA, 20 bp, synthetic construct
  source 1..20: mol_type = other DNA
tgctggtgatgggagttgta

SEQ ID NO: 9 - DNA, 20 bp, synthetic construct
  source 1..20: mol_type = other DNA
cctccaagtagcagccaaag

SEQ ID NO: 10 - DNA, 20 bp, synthetic construct
  source 1..20: mol_type = other DNA
caatgcctctggttcccctt

SEQ ID NO: 11 - DNA, 20 bp, synthetic construct
  source 1..20: mol_type = other DNA
cccctcgaggatttcgacag

SEQ ID NO: 12 - DNA, 23 bp, synthetic construct
  source 1..23: mol_type = other DNA
atgaactttctgctgtcttgggt

SEQ ID NO: 13 - DNA, 22 bp, synthetic construct
  source 1..22: mol_type = other DNA
tggccttggtgaggtttgatcc